European Patent Application EP 4 484 547 A1, published January 1, 2025. Title: Pararhizobium strains, compositions and uses thereof as plant growth stimulants. Applicant: UNIVERSITAT DE BARCELONA. The sequence listing filed with the application follows.

SEQUENCE LISTING (8 sequences)

SEQ ID NO: 1 - DNA, 20 bp, synthetic construct
  source 1..20: mol_type = other DNA; note = Primer 27F
agagtttgatcctggctcag

SEQ ID NO: 2 - DNA, 19 bp, synthetic construct
  source 1..19: mol_type = other DNA; note = Primer 1492R
ggttaccttgttacgactt

SEQ ID NO: 3 - DNA, 21 bp, synthetic construct
  source 1..21: mol_type = other DNA; note = Primer 337F
gactcctacgggaggcwgcag

SEQ ID NO: 4 - DNA, 19 bp, synthetic construct
  source 1..19: mol_type = other DNA; note = Primer 799F
aacmggattagataccckg

SEQ ID NO: 5 - DNA, 21 bp, synthetic construct
  source 1..21: mol_type = other DNA; note = Primer 805R
gactachvgggtatctaatcc

SEQ ID NO: 6 - DNA, 18 bp, synthetic construct
  source 1..18: mol_type = other DNA; note = Primer 1193R
acgtcatccccaccttcc

SEQ ID NO: 7 - DNA, 1446 bp, Pararhizobium
  source 1..1446: mol_type = genomic DNA; note = CECT30825 strain; note = 16S rRNA sequence
tcggttaccctttgtacgacttcaccccagtcgctgaccctaccgtggttagctgcctccttgcggttagcgcactaccttcgggtaaaaccaactcccatggtgtgacgggcggtgtgtacaaggcccgggaacgtattcaccgcagcatgctgatctgcgattactagcgattccaacttcatgcactcgagttgcagagtgcaatccgaactgagatggcttttggagattagctcgacctcgcggtctcgctgcccactgtcaccaccattgtagcacgtgtgtagcccagcccgtaagggccatgaggacttgacgtcatccccaccttcctctcggcttatcaccggcagtccccttagagtgcccaactgaatgctggcaactaagggcgagggttgcgctcgttgcgggacttaacccaacatctcacgacacgagctgacgacagccatgcagcacctgtcaccgatccagcctaactgaaggacaatgtctccactgtccgcgatcgggatgtcaagagctggtaaggttctgcgcgttgcttcgaattaaaccacatgctccaccgcttgtgcgggcccccgtcaattcctttgagttttaatcttgcgaccgtactccccaggcggaatgtttaatgcgttagctgcgccaccgaatagtaaactacccgacggctaacattcatcgtttacggcgtggactaccagggtatctaatcctgtttgctccccacgctttcgcacctcagcgtcagtaatggaccagtgagccgccttcgccactggtgttcctccgaatatctacgaatttcacctctacactcggaattccactcacctcttccatactctagatcgacagtatcaaaggcagttccagagttgagctctgggatttcacccctgactgatcgatccgcctacgtgcgctttacgcccagtaattccgaacaacgctagcccccttcgtattaccgcggctgctggcacgaagttagccggggcttcttctccggataccgtcattatcttctccggtgaaagtgctttacaaccctaaggccttcatcacacacgcggcatggctggatcaggcttgcgcccattgtccaatattccccactgctgcctcccgtaggagtttgggccgtgtctcagtcccaatgtggctgatcatcctctcagaccagctatggatcgtcgccttggtaggcctttaccccaccaactagctaatccaacgcgggctcatccatctccgataaatctttcccccgaagggcgtatacggtattagcacaagtttccctgagttattccgtagagatgggtagattcccacgcgttactcacccgtctgccgctccccttgcggggcgctcgacttgccatggttaagcctgccgccagcgttcgttctgagccatgatccaaa

SEQ ID NO: 8 - DNA, 1438 bp, Pararhizobium
  source 1..1438: mol_type = genomic DNA; note = CECT30826; note = 16S rRNA sequence
ggctcagaacgaacgctggcggcaggcttaacacatgcaagtcgagcgccccgcaaggggagcggcagacgggtgagtaacgcgtgggaatctacccatctctacggaataactcagggaaacttgtgctaataccgtatacgcccttcgggggaaagatttatcggagatggatgagcccgcgttggattagctagttggtggggtaaaggcctaccaaggcgacgatccatagctggtctgagaggatgatcagccacattgggactgagacacggcccaaactcctacgggaggcagcagtggggaatattggacaatgggcgcaagcctgatccagccatgccgcgtgtgtgatgaaggccttagggttgtaaagcactttcaccggagaagataatgacggtatccggagaagaagccccggctaacttcgtgccagcagccgcggtaatacgaagggggctagcgttgttcggaattactgggcgtaaagcgcacgtaggcggatcgatcagtcaggggtgaaatcccagagctcaactctggaactgcctttgatactgtcgatctagagtatggaagaggtgagtggaattccgagtgtagaggtgaaattcgtagatattcggaggaacaccagtggcgaaggcggctcactggtccattactgacgctgaggtgcgaaagcgtggggagcaaacaggattagataccctggtagtccacgccgtaaacgatgaatgttagccgtcgggtagtttactattcggtggcgcagctaacgcattaaacattccgcctggggagtacggtcgcaagattaaaactcaaaggaattgacgggggcccgcacaagcggtggagcatgtggtttaattcgaagcaacgcgcagaaccttaccagctcttgacatcccgatcgcggacagtggagacattgtccttcagttaggctggatcggtgacaggtgctgcatggctgtcgtcagctcgtgtcgtgagatgttgggttaagtcccgcaacgagcgcaaccctcgcccttagttgccagcattcagttgggcactctaaggggactgccggtgataagccgagaggaaggtggggatgacgtcaagtcctcatggcccttacgggctgggctacacacgtgctacaatggtggtgacagtgggcagcgagaccgcgaggtcgagctaatctccaaaagccatctcagttcggattgcactctgcaactcgagtgcatgaagttggaatcgctagtaatcgcagatcagcatgctgcggtgaatacgttcccgggccttgtacacaccgcccgtcacaccatgggagttggttttacccgaaggtagtgcgctaaccgcaaggaggcagctaaccacggtagggtcagcgactggggtgaagtcgtacaaaggggtaaccgga